European Patent Application EP 4 722 354 A1, published April 8, 2026. Title: A composition for ligating single-stranded DNA. Applicant: 国立大学法人九州大学. The sequence listing filed with the application follows.

SEQUENCE LISTING (31 sequences)

SEQ ID NO: 1 - DNA, 1137 bp, synthetic construct
  source 1..1137: mol_type = other DNA
atgctggggaagcctccgttgatcgagaaagcatatcgactggcgaaagaaaccaaggcctttcttattaaacgcaatggcaacctggtgatgtttacgtatgcttacgtccatcccgtaatggcagacccggaagctcgtgaacttcggggcatcatttacgatagtgtgagtggcaacgttgtatcgcgcccctttcataagtttttcaactatcgggaaccgccgttcggtctcaccagggagggttttccggacggggaagtttatctagccccgaaaatggatggttacctccttcaggtgtcattactcgaagacggttcccttctgaaagtcagtaggcgctcactgtcgccgactctgctcaactcagtgttggaagaggtgtggggtgaacgcgaagaggaggcaactcgggaggtgctggagggccttcctcgcccagccacactgctgttcgaagtaacatcttccaaacgaccagtgctggttcgccatcaagcttctgaagttcgcttccttgttgccagagaaatagggaccggccgttatctgctgcccgatgaagtaggctggccgattgagggccagtcactgccctggacccgagtaaggatagatccggataatttcctcgaagaaattaaggatctggaaggagtagagggttacgttgcctttttgccagaaaaaaatgaattcgtcaaatttaaaacaaaatgggcctttagattgtccgggtttctgttagacccagtcgaaggctttgtgtctgcctacgttgaagaccgtgtcgatgatcttctggcaagcctgacagaacggccagatctgcaggaagccatactgagagcaaaagaacttcttgatgggctgtttagcgaagctaccagcttaggagaggagttacgtgaacgcggtattgtacgtaaggaggcgtgggaacaggtcagcagctgggctaaaggtaaaggtttatctgggattgaaggggtgttgaaagaagtagccatggtcgcatatagcggagggcaaacgcgggaagcctttttaaaaggcattggtaaaggtaaatcagtggatttcctgaaaacattagatctgttcccacgcgtaggagaagaagttggggca

SEQ ID NO: 2 - protein, 379 aa, Thermus phage phiLo
MLGKPPLIEKAYRLAKETKAFLIKRNGNLVMFTYAYVHPVMADPEARELRGIIYDSVSGNVVSRPFHKFFNYREPPFGLTREGFPDGEVYLAPKMDGYLLQVSLLEDGSLLKVSRRSLSPTLLNSVLEEVWGEREEEATREVLEGLPRPATLLFEVTSSKRPVLVRHQASEVRFLVAREIGTGRYLLPDEVGWPIEGQSLPWTRVRIDPDNFLEEIKDLEGVEGYVAFLPEKNEFVKFKTKWAFRLSGFLLDPVEGFVSAYVEDRVDDLLASLTERPDLQEAILRAKELLDGLFSEATSLGEELRERGIVRKEAWEQVSSWAKGKGLSGIEGVLKEVAMVAYSGGQTREAFLKGIGKGKSVDFLKTLDLFPRVGEEVGA

SEQ ID NO: 3 - DNA, 1185 bp, synthetic construct
  source 1..1185: mol_type = other DNA
atgctgctgggtccgcccccgccactggatcttgcgctggaaaaagcacaaacgccgccgtttctagtacgaagggacggagggttagtactggtctcataccgcgaacgaggtgcaggtacccaaccttcatgggatccggtcacccgtgagctgagaggtattatttatcgtgaggccacgggagaagtcgtgtcaagaccgtttcatcgctttttcaatttaggagaccccaggtgtggtgtagacccttcaaggtccctgggtccgggtgattacatcggccctaaggaggatggtagattacttcaggcgttttttctggagggcgcattacgttttgccacgcgtgggagccttagactgtcgccagaggatgaacgggcgctgcgccggtcttggacattggatcacgaagcactggccgtaagagcccgcgaggttctgggccctgtcacactacttttcgaggtgctggatccagaaagaccgattatggtccgtccagaagccccgaaagctgtattgctcgcagtcagacatatcccgaccggtcgatattggctcccaggcgtcagtcaggaacttcgtgaagtccttggcggacttagggtgcctcatgtcgtgtgggagcccgcaggttcagcttctctgcaggaagttcaccaaagtatactggaacgcgagggtgtggaaggcttcgtagtgtggctagcacagggtgattttgttaaattgaagacacgttgggctttgggatttaccggtgaacgtggcgatctcgagcgatttcttgaggcatttcgaatcgccttttacgaagaacggctggacgacctgcaggctggcattggagaaggtccgtacagacaagtgtttagctttttaatgtcacgcctagaagatctcgtcagggaagccgtggcccaggccgaggccgtcagaggcctgccgcgcagagaagcctatgaaggtttacgacgcgtcctgggggcaaaacctcagggtctcctgttattaaatgttgccctacgggcgtacgatagaggagaaggcgaagcttgggaagccttaaaacgtgaaatgaagcgggccggacgtggcattcttaaagatctgttagcggaatcggggtttaatgtcgggggcatccctgtgcgcggttggagcgcatttttggaagaa

SEQ ID NO: 4 - protein, 395 aa, Meiothermus luteus
MLLGPPPPLDLALEKAQTPPFLVRRDGGLVLVSYRERGAGTQPSWDPVTRELRGIIYREATGEVVSRPFHRFFNLGDPRCGVDPSRSLGPGDYIGPKEDGRLLQAFFLEGALRFATRGSLRLSPEDERALRRSWTLDHEALAVRAREVLGPVTLLFEVLDPERPIMVRPEAPKAVLLAVRHIPTGRYWLPGVSQELREVLGGLRVPHVVWEPAGSASLQEVHQSILEREGVEGFVVWLAQGDFVKLKTRWALGFTGERGDLERFLEAFRIAFYEERLDDLQAGIGEGPYRQVFSFLMSRLEDLVREAVAQAEAVRGLPRREAYEGLRRVLGAKPQGLLLLNVALRAYDRGEGEAWEALKREMKRAGRGILKDLLAESGFNVGGIPVRGWSAFLEE

SEQ ID NO: 5 - DNA, 1131 bp, synthetic construct
  source 1..1131: mol_type = other DNA
atgcgtaaaccgccgccgccgctgaaaagagcgctggaaatagccgcacatccaccatttcgcgtgcaaagagaggagggacttgtgcttatttcttaccgcgaaaagggtgggttttcggaagcttcctgggatgccgaggcccgcgaattgcgcggtatagtgtacgcggaagcaacgggagaggcagtgtccagaccttttcatagattttttaatctgggcgacccgcgctgtggtttcccgccggatcgccctctgaagaccaatgacttgctagcgcgcaaagttgatggcttcctgttacaggtatttgctttccaggaaaaactgtggtttgcatctcgggcggcgctgcgcttgagcaaggccgaacatgcttcctggcatcaagcctggaccccccggcacgacgcgtttgtgcgacaagcattagagtctctgggtagcattactcttttgtttgaagtggttgacccgaaacgtctgagcctagaacgacacgaagaggcggctgccgtgctgttggctatacgccacatccctactggacggtactggttccctggcgcagccccagaacttgacgctctgctgcagagtttccaggtgcctcacgtgagctggcgcccagcgggcgcgggtaccttagaagaattacaccgtcgagttcgtaatgaaaaagataaggaaggttatgttttgtggctggaggagggcgattttctgaaggttaaaacagactgggcactgggtttttctcgtaaacagcggcggtttcaagatcacctccgtgaattttcgcgctccttaatggaggatcgttttgatgattttattgccggtctctcatccgagccggagatgcagggcgattttctgcgtctttaccgccgaatccggaacttgataggtgagacccttgcgatggcagaggaagttcgaggcttgcctcgaaaagaagcggtcgcgctgcttgaggatcgcttgcgctctttccccttgactcaagcccgcctatctctggccctggccgcctatgaaggcggggaagaacgtgcctgggctcgctttaagactctgctgaaaggtcgtggcccgcagattctggatgcgcttttagaagaagcc

SEQ ID NO: 6 - DNA, 1131 bp, synthetic construct
  source 1..1131: mol_type = other DNA
atgaggaagccgccgcctcctctcaagcgggctctggagatcgcagcccatccgcctttccgcgttcagcgcgaggagggcttggtcctgatcagttatcgcgaaaaaggagggttctccgaggccagttgggacgccgaagcacgtgaattacgcggaattgtttatgcggaagcgactggtgaggctgtttcccgtccgttccatcgcttttttaatttgggcgacccacggtgcgggtttcctccagaccgcccgcttaaaacgaacgacctactagctagaaaagtggacgggttcttacttcaggttttcgctttccaggaaaaattatggtttgcatcaagagctgccctgcgactgtcaaaagcggaacacgctagctggcgccaggcctggaccccgagacacgacgcgtttgtgcgtcaggcactcgaatcacttgggagcatcaccttactctttgaagtagtggacccaaagcgtttatcattagaaagacacgaggaggcagccgcggtcctgctcgccatacgtcatattcctacggggcgttattggttcccaggtgcggccccggaactcgatgccctgctgcagtcttttcaggtgcctcacgtttcgtggagaccagcgggagcaggaacactagaggagttgcatcgtcgggtaagaaatgaaaaggataaagagggctatgttctgtggttagaagaaggggattttctgaaggtcaagacggactgggcactcggcttctcacgcaaacagcggcggttccaagaccatctccgtgaattttcgcgaagtctaatggaggatcgctttgacgatttcattgcaggtttatcttcggagccggaaatgcagggagatttccttagactgtatagacgtattcgcaacctgatcggcgaaacactcgcgatggccgaggaagtgcggggtttaccgcgcaaggaagcggtggcgctgttagagggacgtttacgttcactgccactagctcaagcacgcttgagcctggcgcttgcggcttatgagggtggtgaagaaagagcatgggcccgcttcaagaccttgttaaagggtcgtggccctcagattctggatgctctcctagaagaagca

SEQ ID NO: 7 - DNA, 1149 bp, synthetic construct
  source 1..1149: mol_type = other DNA
atggagcggcctccgcccttcctgcctaaggctttggccctggcagaaaatccccccttttttacacgtcgcaaagacggcttaattctgataggatatcaagaagacggtctggttagggacctggcgtgggatgaagaaaccagagagctgcgtggaattatttaccgggaagcaactggtgcagtgatatctcgcccttttcatcgcttttttaacgtaggggaccctcgctcgggagtagatccgcagcgtcctctggggccgggcgatcttctggcgcctaaagtggatgggcgcctctttcaagtgttttttttagaagggagcctgcggctcgcgacccgcggctcgctcgaactggcaaaagccgaacgtgcttcatggcgtaaagcgtggacagaagatcatgaacgcctcgctcagcgtgcccaggaagccctgggtcctgtcacactcctctttgaagtcgtggatcctgaacgccctattttagaacatcctcaggaagccgcggcagttctgctggcagtccgtcatgtggcgactggacgatatggacttcccggtgccagtgaggttctggaggaactcctgaaaggtctgaaagttccacgtattgcgtgggctccggcgcctcttggggaaacagtcggctcattacacgaacacatccgcaaagaggccggacgcgaggggtttgttttgtggttagccgagggcgattttctgaagttaaagacggattgggccctgggtatcccaaaggaacggggtcgcgctcgcgaattgcggcaggcgtttctggaagcatttctggaacggcgactggatgatctgctgagcgccctggaagacgcacaggagaaaggagcgatggcggagctggccgcaaggctagaagagttgttagcagaagccgttcagcgcgcagaggcgcataaaggccttccgccaaaggaggtatatgttagactggaggccaccctcctgggacagccaatgggtccgcttcgcttgagacttacaatgggcgctcatcgcgccggccgtgaaggcgcctggcgcgtacttgagggcgcgctgcgcgctcggcgtgtctcccttctggaagaactcttagcatctccaccgggctttatgctggaa

SEQ ID NO: 8 - DNA, 1122 bp, synthetic construct
  source 1..1122: mol_type = other DNA
atgtggggtagtccaccgcctctcaaacgggcgctggaactggctgcgcgcccgccgtttcaggttagacgcgaaggtgggctggtgttaatttcatatcaagaaaagggtgggttctcagaaattccgtgggaccgtgaagcgcgtgaactacgtggcattgtttacgcagaagatacaggtgaggcactgagccgtccgttccaccgtttttttaatcttggagatccacgttgtgctttcccaccgggtcgccctctggctgccggcgatctgctcgcccctaaagttgacggacgcctcttgcaggtgttcgcataccgtggcacgccatggtttgcatcacgtggcagcctgcgtctgtcggaggtggaggaagatagccgtagaaaagcatggaccccggatcatgatgtattagttcaacgtgcgtttgcagcgctaggtccggttacgttactgtttgaagtggtggacccagaacgtcccgtggtcgagcgcccaagagaagcggcagtagtactgcttgcggtccgtcacataccaacgggccggtattggtttccgggtgcctctccagaattggaagcactgctggccgacttggatctgccgaggctgtcttggcgcccagctggggaaggcacccttggtgaattgcatcaacgtgtgcggcctgagggtgagcgtgaagggtatgtgctgtggttagcggaaggggactttgtcaaactgaagacagactgggccctgggcttcactcgtaaacgacagtcctttcggaaacgcttacaggaatttgcacaagcattgctcgaagatcgcctagacgatctgctggctggtggtgctgatgaaccggaaagtcagcgtatcttcttgcgcttatatcgaaggctgcagggcttagtagcgcaggccacggcgttggcaggcgaagcccgtgacctatctcgtaaggaagcatatgcacttttcgaagaacgtttagggtctagccgatttctcctggatttagcactacgcgcgcacgagggtggcgaagatcgtgcgtggtcgcgtctaaaggatgtactgcgcaaaaagggtcccgaattcctggaggtcctttgggaagaggct

SEQ ID NO: 9 - DNA, 5327 bp, synthetic construct
  source 1..5327: mol_type = other DNA
tggcgaatgggacgcgccctgtagcggcgcattaagcgcggcgggtgtggtggttacgcgcagcgtgaccgctacacttgccagcgccctagcgcccgctcctttcgctttcttcccttcctttctcgccacgttcgccggctttccccgtcaagctctaaatcgggggctccctttagggttccgatttagtgctttacggcacctcgaccccaaaaaacttgattagggtgatggttcacgtagtgggccatcgccctgatagacggtttttcgccctttgacgttggagtccacgttctttaatagtggactcttgttccaaactggaacaacactcaaccctatctcggtctattcttttgatttataagggattttgccgatttcggcctattggttaaaaaatgagctgatttaacaaaaatttaacgcgaattttaacaaaatattaacgtttacaatttcaggtggcacttttcggggaaatgtgcgcggaacccctatttgtttatttttctaaatacattcaaatatgtatccgctcatgaattaattcttagaaaaactcatcgagcatcaaatgaaactgcaatttattcatatcaggattatcaataccatatttttgaaaaagccgtttctgtaatgaaggagaaaactcaccgaggcagttccataggatggcaagatcctggtatcggtctgcgattccgactcgtccaacatcaatacaacctattaatttcccctcgtcaaaaataaggttatcaagtgagaaatcaccatgagtgacgactgaatccggtgagaatggcaaaagtttatgcatttctttccagacttgttcaacaggccagccattacgctcgtcatcaaaatcactcgcatcaaccaaaccgttattcattcgtgattgcgcctgagcgagacgaaatacgcgatcgctgttaaaaggacaattacaaacaggaatcgaatgcaaccggcgcaggaacactgccagcgcatcaacaatattttcacctgaatcaggatattcttctaatacctggaatgctgttttcccggggatcgcagtggtgagtaaccatgcatcatcaggagtacggataaaatgcttgatggtcggaagaggcataaattccgtcagccagtttagtctgaccatctcatctgtaacatcattggcaacgctacctttgccatgtttcagaaacaactctggcgcatcgggcttcccatacaatcgatagattgtcgcacctgattgcccgacattatcgcgagcccatttatacccatataaatcagcatccatgttggaatttaatcgcggcctagagcaagacgtttcccgttgaatatggctcataacaccccttgtattactgtttatgtaagcagacagttttattgttcatgaccaaaatcccttaacgtgagttttcgttccactgagcgtcagaccccgtagaaaagatcaaaggatcttcttgagatcctttttttctgcgcgtaatctgctgcttgcaaacaaaaaaaccaccgctaccagcggtggtttgtttgccggatcaagagctaccaactctttttccgaaggtaactggcttcagcagagcgcagataccaaatactgtccttctagtgtagccgtagttaggccaccacttcaagaactctgtagcaccgcctacatacctcgctctgctaatcctgttaccagtggctgctgccagtggcgataagtcgtgtcttaccgggttggactcaagacgatagttaccggataaggcgcagcggtcgggctgaacggggggttcgtgcacacagcccagcttggagcgaacgacctacaccgaactgagatacctacagcgtgagctatgagaaagcgccacgcttcccgaagggagaaaggcggacaggtatccggtaagcggcagggtcggaacaggagagcgcacgagggagcttccagggggaaacgcctggtatctttatagtcctgtcgggtttcgccacctctgacttgagcgtcgatttttgtgatgctcgtcaggggggcggagcctatggaaaaacgccagcaacgcggcctttttacggttcctggccttttgctggccttttgctcacatgttctttcctgcgttatcccctgattctgtggataaccgtattaccgcctttgagtgagctgataccgctcgccgcagccgaacgaccgagcgcagcgagtcagtgagcgaggaagcggaagagcgcctgatgcggtattttctccttacgcatctgtgcggtatttcacaccgcatatatggtgcactctcagtacaatctgctctgatgccgcatagttaagccagtatacactccgctatcgctacgtgactgggtcatggctgcgccccgacacccgccaacacccgctgacgcgccctgacgggcttgtctgctcccggcatccgcttacagacaagctgtgaccgtctccgggagctgcatgtgtcagaggttttcaccgtcatcaccgaaacgcgcgaggcagctgcggtaaagctcatcagcgtggtcgtgaagcgattcacagatgtctgcctgttcatccgcgtccagctcgttgagtttctccagaagcgttaatgtctggcttctgataaagcgggccatgttaagggcggttttttcctgtttggtcactgatgcctccgtgtaagggggatttctgttcatgggggtaatgataccgatgaaacgagagaggatgctcacgatacgggttactgatgatgaacatgcccggttactggaacgttgtgagggtaaacaactggcggtatggatgcggcgggaccagagaaaaatcactcagggtcaatgccagcgcttcgttaatacagatgtaggtgttccacagggtagccagcagcatcctgcgatgcagatccggaacataatggtgcagggcgctgacttccgcgtttccagactttacgaaacacggaaaccgaagaccattcatgttgttgctcaggtcgcagacgttttgcagcagcagtcgcttcacgttcgctcgcgtatcggtgattcattctgctaaccagtaaggcaaccccgccagcctagccgggtcctcaacgacaggagcacgatcatgcgcacccgtggggccgccatgccggcgataatggcctgcttctcgccgaaacgtttggtggcgggaccagtgacgaaggcttgagcgagggcgtgcaagattccgaataccgcaagcgacaggccgatcatcgtcgcgctccagcgaaagcggtcctcgccgaaaatgacccagagcgctgccggcacctgtcctacgagttgcatgataaagaagacagtcataagtgcggcgacgatagtcatgccccgcgcccaccggaaggagctgactgggttgaaggctctcaagggcatcggtcgagatcccggtgcctaatgagtgagctaacttacattaattgcgttgcgctcactgcccgctttccagtcgggaaacctgtcgtgccagctgcattaatgaatcggccaacgcgcggggagaggcggtttgcgtattgggcgccagggtggtttttcttttcaccagtgagacgggcaacagctgattgcccttcaccgcctggccctgagagagttgcagcaagcggtccacgctggtttgccccagcaggcgaaaatcctgtttgatggtggttaacggcgggatataacatgagctgtcttcggtatcgtcgtatcccactaccgagatatccgcaccaacgcgcagcccggactcggtaatggcgcgcattgcgcccagcgccatctgatcgttggcaaccagcatcgcagtgggaacgatgccctcattcagcatttgcatggtttgttgaaaaccggacatggcactccagtcgccttcccgttccgctatcggctgaatttgattgcgagtgagatatttatgccagccagccagacgcagacgcgccgagacagaacttaatgggcccgctaacagcgcgatttgctggtgacccaatgcgaccagatgctccacgcccagtcgcgtaccgtcttcatgggagaaaataatactgttgatgggtgtctggtcagagacatcaagaaataacgccggaacattagtgcaggcagcttccacagcaatggcatcctggtcatccagcggatagttaatgatcagcccactgacgcgttgcgcgagaagattgtgcaccgccgctttacaggcttcgacgccgcttcgttctaccatcgacaccaccacgctggcacccagttgatcggcgcgagatttaatcgccgcgacaatttgcgacggcgcgtgcagggccagactggaggtggcaacgccaatcagcaacgactgtttgcccgccagttgttgtgccacgcggttgggaatgtaattcagctccgccatcgccgcttccactttttcccgcgttttcgcagaaacgtggctggcctggttcaccacgcgggaaacggtctgataagagacaccggcatactctgcgacatcgtataacgttactggtttcacattcaccaccctgaattgactctcttccgggcgctatcatgccataccgcgaaaggttttgcgccattcgatggtgtccgggatctcgacgctctcccttatgcgactcctgcattaggaagcagcccagtagtaggttgaggccgttgagcaccgccgccgcaaggaatggtgcatgcaaggagatggcgcccaacagtcccccggccacggggcctgccaccatacccacgccgaaacaagcgctcatgagcccgaagtggcgagcccgatcttccccatcggtgatgtcggcgatataggcgccagcaaccgcacctgtggcgccggtgatgccggccacgatgcgtccggcgtagaggatcgagatctcgatcccgcgaaattaatacgactcactataggggaattgtgagcggataacaattcccctctagaaataattttgtttaactttaagaaggagatataccatgggcagcagccatcatcatcatcatcacagcagcggcctggtgccgcgcggcagccatatggctagcatgactggtggacagcaaatgggtcgcggatccgaattctggagccatccgcagtttgaaaaataacaaagcccgaaaggaagctgagttggctgctgccaccgctgagcaataactagcataaccccttggggcctctaaacgggtcttgaggggttttttgctgaaaggaggaactatatccggat

SEQ ID NO: 10-13 - skipped (4 entries)

SEQ ID NO: 14 - DNA, 103 bp, synthetic construct
  source 1..103: mol_type = other DNA
gtaaaacgacggccagtgaattcgagctcggtacccggggatcctctagagtcgacctgcaggcatgcaagcttggcgtaatcatggtcatagctgtttcctg

SEQ ID NO: 15 - DNA, 33 bp, synthetic construct
  source 1..33: mol_type = other DNA
agatcggaagagcgtcgtgtagggaaagagtgt

SEQ ID NO: 16 - DNA, 33 bp, synthetic construct; identical to SEQ ID NO: 15
  source 1..33: mol_type = other DNA

SEQ ID NO: 17 - skipped

SEQ ID NO: 18 - DNA, 16 bp, synthetic construct
  source 1..16: mol_type = other DNA
gtaaaacgacggccag

SEQ ID NO: 19 - DNA, 17 bp, synthetic construct
  source 1..17: mol_type = other DNA
caggaaacagctatgac

SEQ ID NO: 20 - DNA, 50 bp, synthetic construct
  source 1..50: mol_type = other DNA
gtgactggagttcagacgtgtgctcttccgatccccttattccgatagtg

SEQ ID NO: 21 - DNA, 51 bp, synthetic construct
  source 1..51: mol_type = other DNA
gtgamtggagttmagamgtgtgmtmttmmgatmtcccttattccgatagtg

SEQ ID NO: 22 - DNA, 38 bp, synthetic construct
  source 1..38: mol_type = other DNA
agggagatcggaagagcacacgtctgaactccagtcac

SEQ ID NO: 23 - DNA, 11 bp, synthetic construct
  source 1..11: mol_type = other DNA
cactatcggaa

SEQ ID NO: 24 - DNA, 19 bp, synthetic construct
  source 1..19: mol_type = other DNA
agatcggaagagcgtcgtg

SEQ ID NO: 25 - DNA, 19 bp, synthetic construct
  source 1..19: mol_type = other DNA
agacmggaagagmgcmgcg

SEQ ID NO: 26 - DNA, 19 bp, synthetic construct
  source 1..19: mol_type = other DNA
cacgacgctcttccgatct

SEQ ID NO: 27 - DNA, 19 bp, synthetic construct
  source 1..19: mol_type = other DNA
cgcggcgctcttccggtct

SEQ ID NO: 28 - DNA, 58 bp, synthetic construct
  source 1..58: mol_type = other DNA
aatgatacggcgaccaccgagatctacactctttccctacacgacgctcttccgatct

SEQ ID NO: 29 - DNA, 63 bp, synthetic construct
  source 1..63: mol_type = other DNA
caagcagaagacggcatacgagatcgtgatgtgactggagttcagacgtgtgctcttccgatc

SEQ ID NO: 30 - DNA, 33 bp, synthetic construct
  source 1..33: mol_type = other DNA
acactctttccctacacgacgctcttccgatct

SEQ ID NO: 31 - DNA, 37 bp, synthetic construct
  source 1..37: mol_type = other DNA
acactctttccctacacgacgctcttccgatctnnnn